European Patent Application EP 4 299 727 A1, published January 3, 2024. Title: Novel bacteriophage having a specific bactericidal activity against Clostridium perfringens and antibacterial composition comprising the same. Applicant: CJ CheilJedang Corporation. The sequence listing filed with the application follows.

SEQUENCE LISTING (1 sequence)

SEQ ID NO: 1 - DNA, 51669 bp, bacteriophage CJ_CP_20-29
ctctatcccttccagtctcttcaataatgatgtgtttatcatgtgatacctccctaataagatattttgttatctttggctttctgtcactaaagtccattactgtagctacatccccatcgatgaatactactgatttaccaccaaacttatcttttaagtcatttttattcttgactattttaccattacataaatacatgatatacctcctttaaaggcctctagcagctcctgtaaggtgtctctaccacattataagtaaaatcacattaccacatatctaaaaggccttagaattgattgtgggctcttatatactgtatcttataatatacttcccattaccaagcacttcgtataagaaattgtcatctaagtatatagatcttggttcattagagttagtatactcctcattagtatatacaagggcagctaacttagatactctgtgtatttgttctcccatctccttatcgattgttttagatagtacatacttaccttcttcttgtaacataatgaagaagttagtagtttcaattaatactagttttgtatcagtaaataatgttttcatggttatccctcctttactgtcattataagagaagtaagtacaactgtcaacgttcgggggttctctcttactgttctctccctcgacaaaacaaaatcaagagctcgatcgctgaccgtctgggtttttctatatagggcaaaagctcggaagcatggatatgcctgccgtaatgataatggaggcaaggcaatagcctgccattgatgtaatcaccatgtaatatatatatactatatataataatatattattatatagtatatataatactatgtatatataaagggggcataactgatatccctctacgccagtgataccaatgcctttgtgattttgtagtttcaactgatatgtgggatatcagactgatatggggtaaaaatataggcatatcagatatcagttaatgcctggactttgacatatcagtacaatatatgtataatgtaagcataggaggtagatctaatgaagaataactgggataggttacaagactactttaatattgtaactactaaagaaagtaaagatggtaagcccctaaaaagggaattaaccaatcatgaattgtctgacgcattcgttaaattatatattgaagtatctaaaatgaagagagagaatacccaactaaggaataatatcagagcaatggatggtcatcctgtaatccagattaacgatccgaatgctaaattagatgatatttccttgtatttatatctaaaagacttctggccaagtatatttgaggattataaagccaagatccagagtagtaagatactgaaaggcaagagatttaagtcatttaaagaggctaatgattatgtgtggaaggatctaatccagaatagtaaagtaaagaagactaatgaaagtctatttgtattaagtaaatgggtagatggtatgggtatcaagcataatttcaggaataagcaggagtttgttactgcttgtctgtgctatatggactataaaggatatctggacaaggagggtaagacctttaataagctaggagacatcaagagaggaagcttcagatttaattctgatggggaaacctatgcaatactaaccgatacctttgatattgtgggtaagtataaatctggaattgagaaattcaaattaaaaataaaggagttaaaagagaatgattaaaagaattatgtcattactaacaataattgtgataggagggctactgttaaccatacagagcctaaacaatcattggggaaatgctgtccaagaatatattgagtcgaataaacaattaactgagcagactgaaatactgatggacaatgtagaaggattaaaatatcagaatgataaactgagaactgataaacaaaatctaattgagatgataaattcatttaaaggaatggagttcaaagttgaagttacttattactcatcagatgagcctacagatgtggcaggatatgagaccaagaatagtataggaggggatcttaagattggtgattgggcagctccagactttattcctctacattcattacttcaagtaacatatgcagatggaactcaagagattgcttacatcattgacaggggtaaccctgatgtcattaaggtttttgacagagaagacaaaagaattatacaggactcaacaatgagacttgataagtatgtccatgatgtggatggcaagggagttgatggagcaactataaagatattaagatggggagaataacattctctcttttttatttgacagaatatgacagtatcacttataatagtgttgaggaggtgatagtatggacaatcattcacttgagttcatggaacttcaatctgaatacagagaacttgaaagaagatggcaccaattcctagggggccatgctccttgcgaagaagaagctatccaagttaagaagagaatggaaaagatcaagagaactttacgaaacttgaactaattaaggatttttccagaactcaaaaaattataaaaaggagggttaatccctcccttatttttagaaaacctattgcagtctctttagaactgatacaatatgtcttttctctcttggtgtaaacatccaataataattgtgatttgctttattctcatgtgatcttaatagctttctggctttcctttcatttattccaacctctttggcaatatctcttaatggtattaaattattatctttcatttattacaactccttgattttgttttatagtctatattatgctcagctcggaagatattatacgaattccttcgagaaaatctttgacaaacttccgaggctctcttataataaaatcaacaaataaatacaaaaaggagaactgatatgaaaaggagatatatcgttttacaagttacagttgatgtggattggaaccctgatgttagtgtattagcacataacaaatatttaggagtacactgggtatctgttaaggatgaacacaaggaagatataatctattttgatactgaggaagaagctaagattgaagctaagcatagacctggagctgtagttcaggccacatggaggtagataatatgaaagtaagattagtgattgtaacatcaaaaaggatcttgaccagatattttgaagttgataacaaaagacaggccataggatatattcctaaagtattacaggaggaaggtatatctgataaggttagaaggtatgaagtgattgaggttgatgagaacaacagaagaataaaaagatattaaggggagagatgatctcccttttaacatagaaaggagaattaacatgaaagaatatacttatgtattatgtaagaatgaccagggacaacagtataaaagatatgtggaagtattatgtgagtttgattatatgggcagaaccttattcattcataggcctgtaggagcccctcataatacagtatgttatactatatcagataaggagacaggatgctgtcttgctcctaataactgctctgtaaagacaccttcaaagagatccgcagtaagagtattgaatgaatattttagagaccatgaaatacatgagtgggatatgaagagagtcagaaagttaaaaaaggatttagccagagctccaaagtatcataaagtcaagaaaactccagagcctaaaaaagtaaaaccaaagccagcccaatgtattgatctggattatggtgatatacctttctaaagtttctcttgacatatgatagggaatagtatataataaaattgaggtgataaactatggaaaataataacaacagaataagcagagaaacactttacatggaagttgctaaacttatgacaggaagatctacttgcctaagaaaagcagttggttgtgtattagttagagataacaggatagttgctacttcatataatggagtaccttcaggagtagaacattgtaaaacttgtttaggtcctggatgtgatattgtgatccatgcagaagctggcttaataagttactgtgctaaacatgggatctcaactgaaggaactactatgtatgtaaccttatccccatgtgagagctgtgctaatttaataatcaatgcaggaattaagaaagtggtatatcttgagaaatacagattaagtgagggaatagctaaattaatttgtaatgatgtggaggtagaacaatatgagtaaagaggtatctaatatattagaggatgagaaattaaaggagtttttgagtgaggaacaactagaagctattctaaatatagctaaagctggtaatagtgataaagaagaaaatcttgaggaacttgaaaaattattagaagagaaagaaaatatattaggaggtattaaccatgagtaaaatagtatgtaaaagaagatgttatagaagggatccagcaggtaactgcttagcatatacaattccatatgggccaggagaaaaatgccctagccaatgtaataatccacatcaattaaagaaagagtgtcaagacatcatttctaaaaatcaacctaacaatccaatagtaaaagaatgtctttacttggtagagaagatggatctaataattgggattgagattaataaagcttatgaggaagataagaatagaggttcaggtggaggatctaagaactgtaaacccaatacagcagctctaaagcaaaagatgaaagataatagacctattgaatgtaaacaaactaaagaggagaataaggaatatcaggaagaattaaaacactggcaagaagaccataatgaaaaactagaagttcataaatcagttggatatggtatgaacagaggtaaggtagactcatatactggtatagaacttgatactaaaggtaatccagtatattccccagaagagatacaaattgcagctgataacctgctacaggaaggaagaatagatgtggatatgtatgaaaaaatattgacaggtgaaataaaattataaaacgttgacataattaatccagatgtggtataatagtggtataaatccatagttaattttgccatttggttggtattactagcattaaggttagtgtgccaaccatttttcacgtagtaaagtctggattttaagggggtgatattgtattatgagctataagtcatacactgaaccagagtactgtactcctgaacatttgaagaaagccaaaaaattgatatataatgccctgaaggctgatccctttacacatcctaaacaactaagaaaccttgctaaggtatcacagacctttgttaggcagtgtctaagagagtttaaagagcagggcataacatttttagaagaagaaggtgatattgtggcattgagtagcaaaacaaaaaagactattaagaccctggctgataagtatgatcttgatgagaaagaagagttgtttgtatttcattacatgaagtgctttaatgcaactacagcagctgctagagcaggttatcctgggaataattctcatgcacatgggtctaaactattaaagaagaagaaaatacaggaagctctaaaggctatcagagccgatagagatgaagaattactatgcgatggtatggatgtaataaggcagtacatgaaaatagcctttgcagatataactgatgtgtgccaattcaaggatgatctagttctattaaggtctagtaaggctgtagatggtactttaatcaatgagattaaacaaagtaaagatggcgtatcagttaaaatggaggatagacttcaggcactaaaaagacttgaggtatacttcggcctaagtactgatgtgatgaaagttgaacttgaaaaggttaaattacttttacaaatacaggaaaatcagaataatgctggtaagggaaaagatcttgaggttcttagagccaaaatggctgatagaaagaaaaagaatgcaggtaaaggaaaatctaataccactaagtaaaaaggtattacaggactaaataaagcactttactaaggaggtgtatataattgtttgatttagatagcataattgagaaattagagctagatgctttagttgataagttccacattaacaaggaagctctggaagaaatatcctttgaagaattagtagatctatactatgacgatccttgtggattctcggaagatatactaggagtacacttagatccacatcagaaagatattttattgagtgtaagagacaataagagaacctctgtaaggtcaggacagggggtaggtaagaccatggcctgtgcttgtcttataatttggtatatgacctttaggcctgaatgtaaggtaattgctacagctcctacattttcacagttaacatctgtattatggcctgaaatatcaaaatggctacaaggaactattgtggaagattactttacagtaaataaaactactatgactaggaattgtagtcctatgacttggtttgctatgtgtaaaactagtaatagaaaagagaatatgcttggtcttcatagtgagtttatgctaattatatgtgatgaggctcctggaatagatgatgagatactagaagcattacttggtactatatccgatgaggaaaataagataattttgattggtaaccctgttaaaaatacaggtatcttctttgattctcaccacagtcttaaggaaaattttaaatgtattcatattgacgctacaaaagttgatagaactgataaagaaaaccataaaatgttaaggaaaaagtatggagaagagtccaatgtctacagatgtctggtaaaaggggacttcccactagaagaagatgacatatttatacaattatccacagtatatagaggtattaatagtgaaataaccagacctacagaaccagttactatagatatgggtgtagacgtagctagatttggttcagataagacctctattatgaccaaaattgatggatatgtggaagaacctatctattaccaaggtaaggacactatgaaaacagtaggagaagtgctaagaaaggctaaatccctacatggtgagttccctaaactagcagtagttgtgaaaatagacgacactggtgtaggtgggggagtaactgatagattaaaggagataaaatttgaagaaaaactggactggttgaaggtagtaccatgtaaatttggtatgccattaaagagggggtcccaggcttatgccttttattatgatacaaccacatatatagcctctgtagttaaggaattactggaggatgatgagttaagactaccagataatacagatcttgtgggagaattgactaccagaaagtttaaagtattcaactccaaaggtcaaataaagctggagagtaaggatgaaatgaagaaaagaggactacattctccagacttagcagactctctattcttagcttgccttcctgttggatctaaattaagaaaaatctaagtaactgatatgcctattaaagccaataatttttattctgatatgtgagatatcagttttgaaattgactaggctctatattagtaataatgtgatatagaaggcatatcagagttaccacctttatatatatgtaatataagtatactatatactatataatttatttcataaattaatatagtaatatagtatacattaataattatataattttatatggggaatatatgcggaaaatcttctggaaaataatgtaaaaataaaacgttgacaaatttttgtgaattatgttataataaacgtatcaaattatagttatttttaaatcatgtgaatggccgtatttgacactatatgtggagttgatgtaatcctccctgaaatatgaggccatctggattttataatttgatatataaggtaagaaaggaggtaaagtaactttgaaaaagatatccgccagaagtatatgtggagaccctatccaaaagtctttggatccagtggataaatctaatcaacaaaccagtgtacttggaattgaagttgatgagatatcccctgaatatgacccccaactattagaagtgattataagggagtctacaataataccccaatgcaaaaaggcctaccgaaataatattgctggattcggaataggtattaggtatattgagaaggtagatgaacctactccagaaatggaagctgaatataaacagctggaagaattaattgataccctgtcttttgataaaccaaccaagaatgtctttgaagagatagttgattggagagaaggacttgggtattcttttttagagatcgtagaagatcctaaagactcagctctcgtaaaagagataaaagaaattgaagaccctaagacaattaaaattcttaagctagatgatgagagtacagagtacactgtaacccgatatggtaaacagtacactagaagaaaaagattcagaagatttaagcagactgtaaataatcaatcaatcttctttaaagagtggggagatcctagagatctagatatgaatactggaaagtattatgaaaagggagagatacctcttaaagatcgagctaacagtatacttcattttaaaacaggttatggtgtctatggtacaccaagatgggaaggtcctatgttagccgctcaaggttcaagaaaggccgaattattaaactggagatattttactaatggtaaacatactccattaatgttactaattcaaggtggtactcttaatgataaatcttggaatgaattaactgagtacatgaataatgtaaaaggtgaaaattcccagcatggtttcttagtattagaaactgaagctgcagagagagacactgcccttgatgattctaagccagttactgttgaggtcaagcccctatctgaaatattacagaaggatgagttattccaagactacatggataatactaggaaaaagatacaatcttctttcttactaccagatatatatgtagggtactcccaagattataatgtggctacagccagagaggctacaagaaaaactgaagagcaagtatttgttcctgaaagagaaaacctaacatggatactaaataatgttattctatctggctatggttttaaatatgtggaagcttactttaagagtcctaatattgagaactctgattatcagaaaggaatgtttgctatagcctctagagctatgactcctaatcagattaatgaggagtactattcatcaatcaataaggactatactcctattgatgaagaatgggcaaatatccctacttactcagttgcctcttcaatgagtaataacttaacaagtataattgagaaggctcaaagctctaatgggagtgatgaggtgatagctgtacttaaagaggctaagaaacagttattaaactatcaattaaaaggaggtaagtaatagtgggtactgatgagttgatcgctaaaattgataagatcttaaagaatgaagatgatagccttaagaaagaattgaaagaagctggctatgaggagattgattatacaatagaaaagatctctgaattagaagacactatttctgatctccttacagaagaattaaaacatcttataaaagatggagactttgaaaccattgaagaatttatggaatatgtggagtctcaaataggtacagataatatcgatacttctttagcagaaactcttaagagttgttatcaagaagctatagaaaatttaggagatacttatttacaaggtattgataaggacttatccctaaccaaagtcttttctccatatactactacctttatagatgagtggtcttctaaactaggggaaatgatgaaattaacttcccatgaaaaactacagaatattctggataaggctcttgaagatggagagtctgtagaagatgtagttggtaaattatctgagacttatggctttagtagaactagagctagagctactgctattactgaaatgttaagagctcattcatatgctaaggatgaggcttttaatcaatgccccgcagtaacaggaatacagtggaaacactcagggggaaggggtattcacccaaggcaacaccatgtcgatctggatggtactgtcattaataaaggtgagtacttcactgtaggaatttatgaagctagatttcctagggatatcaacttaccagcttctgagactgtgaattgtcattgtacccatgggcctgtaattgataaggatatactaggattatctaaagaagaaaaagaagctatcagagatcaagtgatagcagaatataatttgtaaaggagggagagtaaatgccagtaaaatcagttaagaaagctattgagatctcagatgctaaaattgattacctttcattagttgataaagcagctaataaatggcaatggattgtggctaaagaacttggggctcctaatagatttagatatgataagccaatcttaaagtctgagtctgaaggagataatcattttgttatcggtgtagtatatgagccaatgactgctgactaccatgataattttatgactgaggaagagatcaagaaagcttgtgagtggtttaatgaaaatggccttggtagtgatttacaacacaatgagaacactcttgagggtgtcaagattgtaaaatcatgggtaactgaggaagatactacaatagaaggtacagtagttaaagctggaacttggctagctaaagctgagattgtcgatgatgatctatggagcaagattgagaaaggcgaaattactggatggtctatgggtggtactggtaaatattctacacaagatgtagatattgatgagattgagaagtctataggtcaatctatacttgataagattggaaaggccttagggttaactccaaagcatatacagaaaggtgcatactctgaaaaatataaagagactgcaaaaagggataatttctggaatgcagttagtaccttagaagatattctatatccatattctagttgggattacactagatcttttgaaagtgatgtagataagataaaggaagctcttcaagaattttctgaaactatggagggaatattattaggaactcccgaggaagtagctaaatcctttgagttaccagtcaataaggcaggtaagaaaatatcttcaaaaaatgtggaaaagttaaaaacagcacaaagtgctattaatgaattattagactcagtggagggggaagaagagatgaatgaaactcaagtacaaaaaatgatagacgaagctatcaaaaaggcattagatggaactaaacctgttgagggtgaagttaaaaagagtgaaggtcaacaagctactactgaagatatagttgctaaggctgtggaaaaagctatgttagaggctggcttaatccagaaacaagaagaaaaaactgaggaagaaaaaatagctgaggcagtagctaaggccatggctccatatgtaggaagtaaacaaattgttaaaaatggaggagaaggacaagaagttcaaaaatcagtatttaatggattatttggtggaaaccaagaataattgataggaggaaaagattatggctaaaataaataaagcagtatttaactctacagtattaagtggtggaggtaaattaaacacagaacaagctaacgcttttattaaaatgataattgatgagccaacaatattaaaagaggctagaactgtaccaatgaaaggagactctaaaaagattgagtcaataggatttggtcaaagagtattaaatcctgcaactgaaggaaaagatccaggggagtctaaatattcagctccaactactggaacagttactttacaagctaaagaatttatagctgtggttaagttaactgatgatactatagaaacaaatatagaaggaaaatcaatagaagacactgtaatgcaattattagctgaaagagttgctcttgatatggaagaaataattgttaatggtgatactagtgagggtagtgatgagttcttacaacaattagatggggttagaaaacagttaactgctcatgtagtagatgctcaaaggggtgctttaagtaaagacctattaaaacaagctaagaaagctgtaccagctaagtatttaagaaaccccagtgagtggagattctactgctcaaatggtttagaaactgattgggtagacttagtaggagagagattaactgctaatggtgatgactcatttataaatggctctgttaaatctgcttatggtgtacctgttaaaggtatagctatgctacaagattatgaagatacttctactcaagtatcagatataatcttaactcaccctaagaatatagttataggtatatcaagagatatcagaattgaattagaaagagctcctagagaaagagctacttatgtagttttaactcttaagatggatgttaagtttgaagatcctaaagctgctgctaagataatcaaggtaaaagcttaatcatgaaggcccactataaatgtgggctctttttcattagaaaggagagatattatggctaaggtcaaattagcaaagggtaaattacaaactctggttattaagggtcatagaattactcaagaccatgtagaagaagttaaagataacctagtaaattatttaaaacagaactatgatgtgattgtcatagatgaacctgttgaggatgaacctctagaagattttactggagaagaaataccttctacagatgacagtaaagaagaacctgctagaagatttacaaacaagaataaaagaaacagataggggtggctcatatgaatattactccggatgaaataattgacttttcaagtaatcctgagattaagaaaagagaccccaaaaatattgagatggatatactaagagctaaagccaagatctcaggaatttttaaaaattcaaataaagactatgatactattgtggagaaaaatcctaatagtaaagaattaaggttagcccatatattgtatgctgagtattatggactacaatccttggtcattagcaaggctgatattcaatccgagacctatgatgattactcatatacaagaagaactgataaggctgtcatagagcctgatattatgcctctgattaaacctttcttagaagatgatagtccatctatcagaacaactactatgagattaagggtactgtaatatgattggaaattcatataacaagctcttaaatcatagatgtaatatataccacctattagaagaccctgaagatcccggatatgggctagcccatacccctagctttagttatcctgatgagccagacatgactgaggtaccctgtcattttaagtcaggaactctagaaaaacttgagtacaaagaacctaggtttaagattacccaggagtactcagtagattttgctattggaactgatgttagacaaaatgataaaattgtggaccttgagactggtatcacatatatagctaaagctcctagggatataagaggtctaaaaattaaggttggtatagaggctaaggattttagatagttatggcttcaaattctggaggcatagaaatagatgctaaacaaatagaaaggtttataaagaagctaagagatgcagctaatagtgatttcaaaaagcaattagcagtatggtttgaagctgcagggatagacttccttgatgtggttcaagatgaaataattagactacaagtagtagacactagattattacttaactcctttcaaaagggaggtaagaatggtatatgggtaagtagtgatggaggactaactttagaagttggtactaacctaaaatatgctaagtgggtaaacgatggtcactacactaatccacaaggacaatcatttagattcgttcctggcatatggtcaggagataaatttatttatcaaccaggagctaagactggtatggtactaagacaaaagaaagtacctggtaaaccttattgggacaatgcagtaaaaatatatgaaaaaatatttgaacaggctttccaaagaaaattagaagattggttagccgaagttttagggggtagttattaatgacagcagatatagggagtattgctaaattcatatctgatctaactggaattactatcctctattttgagcgaatacctgaaaagttcaagtatccctcattatatttcaagaaggtatttaatcctcagaatgatactctttgtagttatagaactgagaatactttaagagttaaggtatttgaacctaaagactctcttgaaattgctcagaatatagctaatgctatatacttgagaaatagaaaaattcctatacttaatagggatggtagtaagaccaacaaaaatctcaaaataaagaatgtggaagtatttgaaggtgaaactgaagaagattctcaggtagagataaactatgatattgtggttagtctttataaagatccaacttacttcgaaaactttgagataacaaagggggtaaaatagtgaaagtacaaaaattttccatacctcaattaagagcccattgtcaacaacttttccaggttgaggagtttgtcttcaacgctgcagttcaatcccttccacctgatgaagagttaacaataaaacaaactagtcagattataaaagactggctaaagaaggaggtaaaatagatggcaggaggaacttttattccaggacaaaataaagtaagacctggtatgtatactagattcgtaagtggtggacttaatgagcctaagcttaataatctaggagttatgatcttaccattacaacttaaatggggtaatgctggagatgttatcaaggtaaccaatgaaggtggcctagaagcattatatcaacttgggtatgacataactcaccctactgtattactagttaaagaggctttaaaagaagctgcaactgttttagtatataacctaacaggtggaactaaagccaaagctgtagtagggtctctaacatttacagctactaaagctggagaaaggggtaataagttatctctaactattaagaccaatcctcttggaggaaaggatatattattatatcttgagggatctaaaatctttgaggctacaggagtaactgaaatatcaacagttaagtctcaatggtttacagtaagtggaagtggttctatagatgagactgctaagactgagtttagtactggtacttctactcagatgaataactctgatgttatcaacttcttagataactgtgagttatacaactttaaaactatggccttcccatttactgatagtgaattacacactgctctattatcaaaacttaaatacttcagagatgaagttggtaagaatattgtggcagttacttctgactttgctacttgtgattacccatacattatcaatgttaagaatggtgttgtattagaagggggcactaagttaacagcttctcaagcaactgcatgggtagctggtgctagagctgcagctggatatactgaagaccttacttataaagcatatcctggagcagtagatgccaatccaagactaaaacactctcaaatagttgatggattaaaaacaggtcaatttatattctcaactcaaactgactcaaattctgaaagagtaaaggtagtagttgaggaagatataaatacacaccatacttttacagaagaatgggatgaaagctttacagataacaaagttgtggctgtattggatgctgttatagatctaggatctcagatcttagttcctaatgttttccctaaccacaaagatggtataaagctagctcaggatagactaataagtctattaactacactacaagctcaaggagcattaaagaatgtggaccctgactctgatgtagtggtagatgaagaagctagtaaaggaaagactatgtatgctactatacttacacaacctgtaagaactttcaagaaatactttgtaactgttaagaataattaaggaggtatagcccatgagtgaagttaatagaatgtctgctagagagggtagagcttttgtatcaggtaagcaagtaactagcttaataaaactagaagctctatttactcctgaggtgactaagaaaagagttatgggtcagaaaggattaacctcaaaagttataggttatgatataactggaactataactcaattcaaagctactccaatgataagagaagctattaaggaatacttaaaaactggtatattccctaagatggatatacaagctgtatgtgatgatccagattctgactatgttaagaattatggtgaggacagagtacaattactaggagtacaattagaaggagatttaccactaattggactagatgctgagggagaagaaattcaagaagaaatatcattctcagcttcagaagtaagatatttataaaagattaagaatattgtggaggtagattattatgtcaaaatttagtatggaatttttcatggaaaatgataagggtaaacaatcacccgaaattgaagttgaaggggtagctagatttagtttccctgagggtcatgaattagcgggccaacctataccttggatattaaagccaatcactactaagcaaatggaagatatccaaaagagaaatacagtaattactagaaacaaaggtataactaactcaataacagaccaaagaagagctactagggaaatgatactagaaacaatagtattccctgactttaaagatccaaaatggttagagtctactaagtttgtggatccagtagatttacttatggatgtactaagcttaccaggagatttcactagaataactagtgaggttatggacataaatggattaggcgataataaggatgatctaatcaaagaagcaaaaaactaataaaggccgacactagtgcattttgggctcatgtgttattccagaagcataatatactaccctgggaatttgataaactatctcccaataggaaagcctttcttatagcctcatgtgaactggctttagaggaagataaaaaagctagggataagttaaagaaaggctcttaatcataaaggagggatataatggcaagtcaagcggcatttactgccatattctctgcccaagataagatctctggtgcatttaaccagatggctgatagtggtaattccttcatgggtactcttgccaaaattggtggagtagctgctggagtattctcagctaaggctgtctgggattttactaaggacagtgttaaagcctttggggattttgagcaaggtttaaatgaggttatgactctattacccaactctactcaagagacctttgataagatgtccggccaggtaaaaaagttaagttctgatatagggatattgcctgataaagtagtacctgctctttatcaagctatatcctcatcagttccagaggataacgtttttagtttcttagaaacagctggtaaagcttctataggtggtatcacatcaatagaaactgcggttgatggactaactactgttattaactcatatggagctaagaatatggatgttcaaagggcctcagaccttatgtttactacagtaagacttggtaagactaactttgagcaactatcacaatccctattcaatgtgctaccttcagcctcagctgctggggtatcttttgaagaagtatctgcctctatagctgcattaacagctcagggggttccaacatctgtagctactactaagataagagctgctatagatgagctatctaaatcgggaaccaagactgataaagtcttccgggaaatagctggtaagggcttcaaagacttcattaaaggtggaggtaatatccaagaggcccttcagatgttagaaaaacatgcccagaaaagtaatctgggtatcaatgacctctttggttctgtagaagctggttcagctgcactagccttgactggtgaaggtactgaggcctttactaatgctcttaatgagatgaaggatagtgctggggccactgaagctgcctatgaaaaaatggataagggctttaatagaaccatggagagaataaaaaccaaagctgctgtagttatgttagatgtgggagatgccctagcccctgccgttgaggttatagctaatgctgttctaaatggtatcacatttatacaagaaggctttgaaaaactaggacctatattctcaatggttgtttctgctttccaaggtttaggagagactatatattacatcatgaatggttgggagtttggggatgctatgcaaccctttatagatctaaccaatgatatattatataagttcttacctgctgatgtggcagatcaaattaatgagaagatatggagtcttggagaagacatctataataattttggagagatcttaataggtctaccagattatttatcagaggctaataataatatacaagaagcctttaatggtttagctgagcctatcatgggagtattagctcctataggtcaagtacttcttgatatgtttggaactttagcttctatatttatgaataacctaattccagccatagacttagtagttctttatgttcaaggctttactcaagtatggcaaactgtattggaagtgttaggccctatattagaagtattaggttctatgttctctgctacttttacagctcttggagaattgataactaatgttttcatgccaatagctgtatcattagctgaagcctttaacacctacatagccccagctatatcacaagttgtggaagctataggtaacttcctaatgccaatattacaaggactagcagattggtggaataatacactactacctatgttcttaagctttgctgagaatgtagttccatatattcaatcagctattgagagttttggtatgatattccaagggttggtggatatgctaactccactacttaaccttttagccgcatctttccaaacagtatggcctgttatctcctcagttgttactggggccgttcaaactatatcaggaatactacagggattaatgcagatgttgagtggtttaatagcttttgtggctggagtattcacaggtaattggtctaaagcttgggaaggtgttaagaacatctttgggggtattttccaaggtatgttatccctagcaaaagctcctattaatagtattattggtatgattaataacttaattggtgctcttaatactattaagatacctgactgggtacctattattgggggtaagggtattaatattccccagataccaatgcttgctgaaggtactgacttctttacagataaagctgccatggttggtgaagctggtcctgaattagttatgggtcctacattctcaaaaatgcctagaggctctcaagtattacctgcagataaaactcaggatttactaagacaatctggagcaggaagtgatgatggatctaaagttatgaacattaacaactcatttaatttcacagtacaggctgaagatggaacaatctcagaaagtgaattaatgagagtatacagatttattgtggaaatgttaaatcaggaaatgttcgagggaggtgaactggaccttgcatagtaaatatcaattctggttaatacagggagatactaggtttaggttaccagtaaatcccactgatataaatatctctgatagtagagataatagtacagtttccattgaaggcttaggggaactctctttcataggagaccctaagctaaaatctttttcttttaattttgagttaccaagctcatactacgatggatgtgagtatactgatattgcagaccctagagtaagttatgctaaacttattgaaatgggtaaagatccagtaagatttactattactagtactgatattaacttattagttactattgataatatctcatatactgagaaaggtggagatattggtactcttcaagtaaaaataaaactaactgagtataagaagcctgaggttaaatcagttagttttacaattccaaaacctaaactagcctatagtggtaatacaggaggtagttcttctggaggtactcaaccttgggcagctactactactaatgtttactcatggctatgggtaagaactggaccaggtatcaataatcccactaagggtaagatatggcctaatgaacactttacagtattaagatctcaaaatggatggcattatgtaaagtataaattagataatggttcaggatataaagaaggttggagttctggtgattatataaggaggttataatatgcaattaattgtggtacaaggagataaatcctttgatattacaaatacctccagtggtaagagttgggcagggtcttcttcatctgcccctcgtaccctatcattccaatataatgctcaagatatacatccaatttatgatggagatcaggtagtactagtccatgagggtaagaatatctttaatggtattattatgaatatctcagataatgagaaaaagcatttacttaaggttaaagcttatgaccctatgatttattgggctaataataaagatagctttgtattcgaaaaccaaactggcgaagctatatttgagtcattatgtaaagcctttggggttgcccctggagtagtagctaaaactggatatactttctctagtttagtatgtgagaaacaaactccctatgatattatgaagaaggtaataaaagaggtttatgaacaaactggagaacagttttatatttactataattctattacaggtaagtttgattttataaaccgaagaaccaataatgaattgtggaaattcgaatatggtaaaaatattggaaccttttcaagaagtagaaactttgatagtattgtcaaccaggtaaagctagtatgtaaatataaacagggtaagggtaaagatgatcccgagattactttatttgcctctgctaaagatgatagcagccaaaagaaatatggtgtatttcaattatacgatactatcagtgatgaactaaaccaagcccaattaaatgagaaggctagaataaagctagaaacaggtaagagacctaaaactgatatctctataactgttataggtgtacctgattgtattagtggcaaagccattgtggttagtataccacatttaaaaattaacaaggctttctacattgagtctgatacccataaatttgatactgactacaccatgaatttaaaacttaaatgtactgaggagggtgatatttaatggctaataatttattagactgtgtaaaacaagtatatagtaatatgtccacccctctaaatatttatagagctaaggtacttagtactagccctctaaaatgtgagtgtcttcacaatagaaaattagtactatctggaaatattatagatgttccaaaacatattgagtctattagtgagggcgatactgtttatcttatgccctatgatgatggacaaagatattttatgttagggatcttaggaggttgatataatgctacctaatggctttaaagatactcttatagttgatgagaaaacaatggagaataccaagacctataaactggatctaaaccttaataggatttatgataatgtggatggtcttgaggccttaaaacaatctttatataaaagattaataactcctaaaaatgcctatatgatttatcaagatacttcttatggttgtgatattagagctttgattaatgactctctagtaactcctgaacttcttgaaatggagattaatagggctatccctgaatgtctcttagaagatgatagagtgactaaagtaactgatctaaagtataatgtgcaaggtaagaatgtatatattgaagtatggataaataccatatatggagatacaaaactggaaggggtgatataatgggattttctgaagatttattctcccgaacacataaagaattattagaagaaatgataggcctatcccctgatgatattgacactagaactggaagcttcacctatgatatggctatggtttttgctgttaagctagctgagttttatgctgttaatgttaatcaaatattagactcagtatttctaagtactgctacaggtaagttcttagatgagagagctgccaatgtagggatatccagaataattccaactaagtgtagaaggtcagctatatttgttggctatgaacccgatgttggttcaagattccaaggaggagattatttctggcaagtgatagagcctaatattattgaatgtgagaccttaggttcaggacccaataaagtatcaacaggtacacatttaattcctatcaatgctatagcagaacttagaagtgctactatgggagatatacttgttattggtagagatcaggagacagatgatgagttaagagaaagagctactaaagccactatacaaccatctggagatgggaatgttcaacagttaactgattggtgtaaaagtgtagctggagtgggtaaagctgtggttcttccctgttgggatggaataaatactgctaaaggtattataaccacagttgaaaataagcctgctaatcctgagctagttaataaagttcaagaatacatggatccaggcaagaaaggtttaggtgagggtaaagctcctataggatgtgtttttactgttgagtcagcccaaacctttaatatcactgtaagagctcaagttaagaaattgagttcagttacagaagaacaaataaaattaaacttcaagaaagaactagaagaatttctaaatagtcaagtatttaaaattactagcctatctataaatagaataggggctatgcttttaaatattgagggagtagaagattatacaaccattacacttaatggaagtagtcaatctttaactattcctgctaatcaaataccaaccattactgaggtggtggtaacttatgtatagtctagaacaggttcaaaaagaattactattgtatgttcctgaattttatgataatataaaagaggctgataacttagtaaacaccattatggctactgaacttcagaagttatatactaagggacaggaattacaagactatgtggatcccaagaccactcctaaggaaggtctagaaagattttttactgatcttgagttatataaatactttgattacccaccaactgaccaagagaaaagagctattattacagtagttctatctgcttggaaaaagtttaatagtacatctatcaaaaatcttactaaggcctatacaggtggaaaggtaaaggtagagttcatagctgaagagagtaagatcaagattagctttactgacctaccaggggtaccacctaacctaaaggctctagaaagagtattcaggggaagaatgcctgctcacctaatatatcaaattatattactttatattacttgggagatgttcgatagatatgattatatgtggagcaagtgggacagtctagatcttacctgggaaaaatgggaagaatatgctataactgaataaaggaggtatgcaaaatgccaagtactagtaaaactcctaccctaggtttaaataagtgggagttaacagataagccaaaaatgaatgattttaacaaggacaatgagaacattgagaactttgctaccgaacataaacagaaaatgactgaggtagaaaagaagtctaagtctaatgaggataggctagatgctttaagggttggtactattaataggcttgagtggtacaactctgagtcttatactggtcctggtaatatcacacccattacagatactccaacccagagacgaggttttaaatggtctggtatgtcaacaggtccacaaactcttgagattaaaactctgcctatagaaccaaatagtgattatatactagcctttctagaagatattgaaggtagttttactagctatgaaattaaactggcttacactaatggaggtcaacaatataggagtattgtaaaacaaggtagtacaccacagagtaatgggtacaagttaaaaactcataaatttagtattccatctggagctactgataccaaaatacaatttgtggtacagagtgcaacctcaagtacctcattaaaggtactaaacctcatattagctaggggtaatgtagtacctgattataatctagcccctgaggatgtgctaaaaagattagacctattatttgagaaagacaccagtttacaaaatcaagtagaccgaaaggctaatcaagatcaagcacttattaaggttagtgctcccttagatagagattgtaattcctttaaacaagcgaatgccttcttctactttgatacaggaactggtgactttaaaaatacccccgagggaaccttagcccatatgagtaatagggtttttatggttagaaatacaggtgagaggggattccaacaggagtttattaacctatacccaaccaataaaataactagatatgttagaaactacacatcaggaaataattcttggagtaagtggtataaggtttatgatgaggctaataagcctacccctgctgacctaaaggcttatcccattcctaaggacgccataactgattttaatacagctttaactgaggggcaatacctgatctcaggtgagttacctaatgccccactaactggtacaaaatatggtatactgatagtatatgttagtacagagactaagcataataatactaataactggatatggcaagggtattatgatactaatggtaataagtattggaggtataaagtaaataatacggattggttcccttggagaaaagattataactccggagctaagccaacacccgcagatattggggcctgggataaaacagccaaaagactagagggtgtagatctaaacaccattacagagggaggtatttattctacagttagaaattctgtcgatagaaatgccccaatcctagcagatgggagattgattgttttatcctggaatacaggacactgggcttctcaaatgttctttgcagatggtggaagagtttttactagaacagctacaaacattgagggtaccggatggacgaattgggctgaaatatatagtaaacaaaataagcctactccagcagatattggtgccttacctactatgggtggagaattatcaggccatctaatcatgagaccgggtcagaaatttattggggcccacaattatggatttagctgtaggactaaagaaggcagtgatgactatgtgatctatatagatgcagataataaagtccatatagggtatgctggaaggcctgtaaagatagactctctggatattgttaataagaacaataagaaggtctatcatgaagataataaaccaactgcagcagatgtgggggcatccccaactaaccatacccatgagggagtttatttaactattagaaaagatgatatagtagattttaatctttgtaaggaagaggggatatactcagtatctagtgtagataccttaccaaactcccctgtagtttacacatatggtatttatggaactctattggtattacccaaggggggtgaggtaactcaactatttacagatagttatggcaaaacatatactaggttttgtagttttaaaggcatatggtccgaatggtgtatagcttatagtaacctcaataaacctaagccatccgatataggagctgcagcctcagaccataaccatgatagtgcttatttaggtaaaaccgctacagctgctaacagtaataaactaaaagaatgggacttagctggagctagtaatgactatgcaggtatcccttttatatcacatgatggagttatggaactaggtcctatattagatttccacttaaagggtagtaagaaagattttgatatgaggataactactagagacggatctctagaggttgataaggctctatcagctgaaaacctatgggctagaaaatacctaagaataaatgactggtatggtggagctgaagatggaagattgtatttcaaacaagagaacaaaaagctatatactgagaatgttactgacttcgttgtaaataatagatctattgctaaaggagattattgggataatgacaatggtaacgttagagtatgtcatcttgggggaggactaagattagtccgtcaaatagttaagacgggttatgctaactcaggtggaggtgtaagttatactatacattttcctaaggcttggaattgggtattacctatatctctagtatcacataactataatgacgcttctaataatacctcaggttattgtactattgactattggaataactcatatttgaatggtggatgttatcaaatggtagctggtaagccaactcaaataatactaacctatttagccactgagtaaaggagttgataaaacatgagaatagtaggatttaattattctgtggaaactaataaaatcatagaccttatattctatgatgatgaaaaagaaatgctgataaatcaggcagaagactcagaagatgtaaaatcatttatagataaagaccatgaagaagttactaagatattagacctaattaataggcctgaacctctatactatagagaggatagtgaaatattaaataatatagaagatattatatgtctccatatacctcataattcacaagggcatttagcctttgtggataacactgaggtaattgatctagacaatctttcagccatacaaatgactgtaagtttatttgaccacataaagggtggcccaaccaaatttgatattagtaaaaagagatcagatctatacagtatcaaagataaggacctatttacttcctatgaggctatagatcctaatcctctggatattaataaattaattggttatcaagcccaggctcttgctgatactaaattagagctaatgcaaactaaggccataatgaaagtattaacacaagaactagctgatataaagattaaaatgatgaataaataaggaggtagggattatgaatttctgggaaatggcttatagaattggagcaataggtaaggacaaattacatcaggcggtaaaatgctcttctaatccggaaggagaaattacaccagaggactataaaagaatatgtggtgaagactttaaggaaagggtgtaatctatggaaaaagaaatactaactcaagttcttagccaaggtatcttttgtagtctatttgtatggctattatatgacactagacaagaagctagagaaagggagaataaattaaatcaagtgatagataagctagttgataaattcaaggtagttgaggatatcaaagaggatgtagatactataaaagatcacctatttagtaacaaaggttaacttataagcctagcaggccatttaaggcctgttaggttttatataaggaaatatattaaggaggtggttaaaatgctgtagcgagcctctcaggcccaataaaacactataatatataaaggagatgtttattatgaaaatcaataaaagattaagtactacgaatgttactctaaatgcaaataatcctgggtatataattatccacgaaactgataatacctcttggggtgctggagccgaaacccactgtaaggctcaagcaaatggaaatataggtaaagccagtgtccattattatgtcgatgatacaggggtatatcaagctgtagaacacaaacacgccacttggaattgtggagatggtcataatagatacggtatcaataatagaaatacaatatctatagaaatatgtgttaatcctgactctgactacaataaggcagttgataatgctgtagagctagttagatacctaaagaatggctactattctaattgtaaagtagtaagacactatgatgccagtagaaaaaattgtcctagaagaatgatagccaatggttactggaatacattcctagaaagagtaaattcaggagagagctcaagctcaccagtaatcaataaccccaaaggattctatgagtctaatgagacaagaactaatgctactttagtgggggaaggttcaatagaagttctagatgaggattgtaagccagtccctggtagatttattgatagcctagataatttatttgttctcggaatatatccttctagaaatttcatagaagttgtatatcctggaaagaataagaagtaccatgcttatattgacataaaacattacagcagattaagttttgactaccacatgaaatatcaaaatgacaatggagtaacttatgtgtggtggaaccctgaagacgttaacatcaaagatcataatgaagaactacagcctggtcaaaaggctagcccaatgtatagaactaatggctggttaagaataacattttatagaaaggatggtactccatctgatggatacgttcgctacgagggtgagcaaagccagaaattctatgaggatgttaaacaaggaatagttaaagttaacacttctcttaatgtaagagatgatgtgaatggtaatataataggctcagtatttagtaatgagagagttactatattgggaagtaagaatggttggtatcatatagaatataatactagccacggtaagaagcaaggttatgtaagttcaaaatatgtagagataatttagggggtatttatcatggaagaaaatttagtaaacttaatattcaattacattgatccacagcttttaataatcattgtatcatgttactgtttaggtctgtttatcaaggctaagccttatataccagattggtctataccattaatacttttgatattcagtatatcattatcaatcttatatatggcaattcaattagaattaggttttacagccaagacctttttgaatggctttatacagggtttaatatgtgcagctgtagcttcctttggtaatcaagtatggaagcagttaatggataagagaaaatcagatcctcctgtaaatcaataggggatagaggttgggcctactttatttagaaagtaggtccttaacctttttaaattcttcttcattatcccattcccattgctttcctggttttacaacctctttgtttcttaagatccttcttgcctttttaccattcatatttaattcttcaagtatcatctttagtgtaaatacaccttctttagtttttggttttttcttagtttcaaccttttcttcttcaggttccttaacatctgttagatcaagagtaattttagtttgttcagccttttcttcaggttcagctggttgttgtacctcttcaactttttcttcttgtggttgttggatttgttggatagcagctattagatcagcctttttcatagtccaccagtttttaacttttaattcctttgctaattctttaatttcaacagctttcatagtatttaaatctttcatatcatttacctcttctttcttatttgttttatctacattttcattataagagatttcctctggtttgtcagggatttcttttaataattttggacctccccagttacattcttctccatcagcattatcaaagacctttcttccttcttctgtgtaacctattacctctccatcagcaaatactaaaccttttttaacaagtgatgagatcacacctctagccttagttccttctatacctgagttttctattactgagaatacccatacacagtcaacatctagtccatcatcaaattcattctttctcatagcatttaatatctttgtttccattgcagttaagttcatatttaacatctcctctttgtttttgtttacaagtttattataagagttattgccagagatgtcaaaggttttctccacagatttataaaatttctttgagatcttagttggtatcacatatttaaagcccttacatttaaagcaagtagtgttaccatctgaggttcttgagtaatggccagtgcctccacatctagggcaagttttaagtaaacccttcttagcaacctttgacatagtgctagcccatatcttaccaaagccatatttgattttagctttatctgaaagatcagggtacaccatattaattatatcaccctttaatggatcatccttgatataactattataccaatctaatttaacctgtgtatgtgatctcctacttattaccttagtaacctcatactcctttaaccacccatctatggcctcattggataattgatcagcctcttcaaaagttatgctattaacaggtatactaaatgctcctgttgctacccagcttccatcttctttttgacaaccaaagaagttttcagcttctacttgaatactataatatatatctatcatgtgatttaccccctaagttatttgttaatataattataccagcactctcgagatatgtcaacgaaaaaagagaagaagtttaccttcttcccctaacctttaagttgattaatagatcatatatatctttaggcataccttgctcccactcccactgtttaccaggtttctcaatattattctttcttaatatacttctagcctttcttggatctagttctattaattcacataaatcttttaaagtgtatatatcacttctagtttgtgctacagctgagttttcaccttttctagcctgttgcactttgttgtaataaagactagttaattttttatgtaaaggactatgtgaccaataagttaagtgagccaattcatggcatatagtttcaagaacacagtccttaatatcccagccaaattttttgattttatcataagctttttctccttcctgtgcaaacctgaaagggaaaaggttaattgtaatcccagtaaatttattacctgatctatggcatagaccatagtagttagcatccacatcagattctatataaagatcaacagcacttacaccaaatgcttttcctaagatcattgtggcctcattgtataactcctttacctcatattcagctaattgattttctatcatatctctcattttgtttacctccaatagttaatttatgatttaattataagagagaactctggatctgtcaacgaaaaacttcgaagaaaaaggatggggtttaccatcctagatcatcccttcttcctatatcatatattgcacagatgcaagcctcaagatgtttttcaatctcagcttttttatgatgtttacatacataatatttagttactcccatttgttgtagtagttctatcaccttatccaagaattgtttttggaagttcttttcaaaaaccaccttatttattttttctatctcatttaacatttctaatttagtcatttttcattcctcctaagaattaattaatattgattacaatattattattataccagagggcccagactatgtcaacgagattctggagattttttcgaaaaaaatagatggccttttggccacccatattaattggcttttttcatttttagtataacctcttcataggcaaccatacagcaagaaaggtagtctcctaattcactttccctaactttgttgcttagtccaaaggattttacctgtttatctagttcttttctaaattgtggatagattttattatccatagccttttgagcaattccttttattacattaagtttttctgatcttgttagttccatagttaacatctccttcaattaattttgattacaatattattatactagatagtcccgatcctgtcaacgattaaatccagatttttagaaaaataaaaaaggaggtttttacacctccttagttttatagatccttgaacatttcagggtagttacataaagtatcttccacatattgttctgggtggtaatcatattctatgatgtattcaacagcagctattaagtcattctcatcattaaattctaccccttgtatttctagttcctcctttaattgttctaaagtttcttgaaattttttgttattcataattaacaactcctttgaattaattttgtttacaagattattataccagactctggagtctatgtcaaagaaaatcccgaatttctttttggcatgaaagttgctaggtatcggatcgctttaaaaagaagcaactatttagttgctcccactggggttaatgaaaaccctgatagttttttattctttccccacctagcacaagattccattgtgggctcaatacccaagatattgcatatatccaaatattcttttaaccataataacctcataataactaatcctcctttgagtatcttaacttcttagattttttattcttatacatcattgagtcggcctgtactatagcttcttcaatagttttacctttaccatagccacatgatagctcagggtatatattcaaggtattgcacagattataagctatatcactgataactacaaactcatcaccaccccctctaatcaatatatccttctcaggatgtaaatgggccttaataagatttaccgtgtattgtatatacacatctccttctagatgacctaatttatcattgaactcttttagatcattaagatcaatatatacaatctcatactcatcaaggtcaatcttatagtttctattataggctcctgtccaatcaatagataactcctttacaagttcaatcaattcttcccttgtaagtttttcaagatctttcatattcagttctctccttttttgtttgattacaatatttatattaccatatactgtggatattgtcaacgaaaaagaagaggtttttaaacctcccccttattttaacattttcttaatatcctcaagttcagatcctgaccatttatagggtttgtttacaccttgctttcttagcttggccctggctttacttggatctaatcctaatgactcacataaaatttttaagtcaactgttcccgtaggtgcattacctccagaaggtgtagggtaagttcccttagcctcaactttattcagatcaaccttctttataggtttgtcctttttctttcttggcttcttaggctcatcgggattaaattctttcattaattctctctccttcttcttttcctcatttaggagtcttaacctttcaagtcttttttgttttttcttttcctccttgactttaatcttggttagagctttaatagttttaccagcctcaattaaagccttagctatttcagtatgattacttattctaggttgttcttttctcattacttatcacctcaattctatattaccacattacttatcaatagtcaacagtttttctgctctatcccttttaagctgtattgattttaatattttctcatcaatagtattctccgttattaagtgtattatttgccaaggctccttttgaccattccttttgattctggcaatagcttgcacataatcatcatatttatagttccaactatagaatattaaccttgaggccctgaagaggtttagaccaacactacctgagcttatttgtagtattaatatatcaatcttgccctcctgaaaatccttattgatctcagctctattcttagtagatcctgttaagcattctactctgtgggtctttttaaaagtatcatgtataagttttatttcctcaagaaaattacatattacaacaacaggctttttatatccttctagatagtcctgtaacaagcctaatttgcctttatcaatattaatattatttcctacattgtttgtgataaatcctcctgagatctgctgtagcctcaaatattgggtaatagtaagatcagctgttaattggttgataaacatattagcccttaagaataaatcctcatagggctcattactctcatagggtataccattagaccttaataaggcctttaattgctttctaggaatgttttcctgtactatatctagttgtgctatcatttcctttctaaggtcattataggcctttctggctttactatttaattcacaggttaaatacagatcaggaagttgttctggtaaatcaatacaatcttctattcttactatatagcaattctggtgcataaggttctttaatatttcctcattcttataccccacaatttcatagttcatataacctcctttgattataaagtcatcttcaaactgtttccaattaactcctagaatatttgagttcataattttatattgcataaataaatcttcataaccattaggagtgggagtccctgacattatcaacctatatttacatttagtagcaattttatatagagccttagatatctgggcatttctattctttaccttatgggattcgtcaacaacaataaactgtggctttaagttcataaggtatttatccatcaacctagccttctcaaaattggcaataataatctttaatcctgagtaggattttatagctctataggtttccataaccttggtcttattaccctgtaatttaaatatcctatattccttaagtttagtaaatttatggatctcagactcccagttaaatacaatagatttaggtgagaatattagtacagtatctagaccttcaagtttctcaagggccacaatagggactaaggtcttacccgtacccatgtccataaatagggcaaacttttctttatttaaaaatagttgtaatgcttctttctgatgtttaaataattttctcttcatactaaaaaagaagaggcattaaagcctcctccttatacctccttagccagttttacaagttcatctcttgaggccttactatggaatttaaccccattatcttttagatattgttttaaggattctttattcatactatcaaaatctaattcttcttcgtcgtaaacattgtcatcatcatctaagtcatcatcgtcattatcatctaggtcttcttcatcatattcttctttactaagatcatgtatttctgagttatcatcactagttagttccatagcagccataatggcatagttagctaggtctagtaaagtatcaaccacagattctttttgagcagcatatgaagggaagtcatcttgatctcctagtaataaacttttagctcttcctagcttatcttcaagtcttatacatagaacagggtttccatattcaagataagtcttgtggaaattatccccatatagattattctttaattcatacagatctcctagttctcctaggaattgttggtgtctttctaaatttttcatgtaatctcctccttgtatattcagctgaggtagccataaaagctattcctcctgctagatttattttatttataatgtctttttgtttttgagttaggttcttttcttttccaggaagtttaacttcaataccaataaacttacctttgtggcaacctagtatatcaggtaagccagctatttgaaatggtcccccatgagttttaaaccaaaaacctgggtattcttttttaagcatattcattatggatttaaccacatctctttcaagcataatagtagcctccaagggtaaataaaggaggaccttaaaggccctcatattttaataattaaattttattcttcatcatcttcttctagcatttctatgatgtcatccttagacattccttttttaacctttaagcctctgtccttagcttcagctttaagttcttttaaagtcattgactcatagtcattttcttcttcatcttcctcttcttcatcttcctcttcttcatcctcatcttcttcgtcatcttcatcagagtctccgaataggtcattatattgttcagctatttcttcttcgtcagcttcttcttcaattagatcaattagatcttcttcagttttagccttcttgattttcttagctgggatttttaaagccttagctaattcttttagctcatccttgtctaattcttcaagatcaacttcagactcatcgtcttcatcatcttcttcatcatcatctgagtcatcatcctcatcttcgtcatcatcagagtcagcttcgtcaaggtttataaaatcagttattcttgatttcttcttaccctcatatatttcatgtgatacttctaccccacattgtaaaccaactagagcttctgtatctaattcgaactcctcatcagggatatcaaatcctaaagcaactaacacaccttttaagttaaataaagcttgtggttgaagtgagcaaatgtggtataacttttgtcctttcatctttccttctgctattacaaaagtaaatgataaataattgcttccactattttcagaaaccttaacctctacatcttctacttccacaatgtaatttccttctgggatagtaactgaagtttcaacgtttgaaagatcaatctttaatcctcctttgtttttgttacctctcttagtagtctttttagccatgttattgtcctccttaaattttaaaatatcattatgagataaatatttgtcaagatattgtacctctttgtttacaagtttatattatcagatttttaattggttgtcaaaggtatttttagaaaattttattttttctttttaccagatttcttactggtttttttaccagatttagctggcttattattccattcaccagccagaatagtttcaatatcctcccagatagttgttggtgattttaaatcatgtaccagataagctggacattcagatccttgaggtctagtaaatttagtaatataataagggttaggtcctagtcttagtctatactggatttctttcttaaccttcataccctctttttctgagtgttcatataaataagtatgacctattactcttgatacagcacataaatatttagatacagatggcattaatcctggtcctacctcaggcattaattggtcttctccttcaccatcaccagattctaacctatcttgtactataaagcatggtagtataccttcctcatttaattctttataaaggtttataacctctttcatataattagccacatttccaaacattctttggctcatctggtccttaccttcttcagctttgaccttttcattacctaattcttgtaaagcagttaaatggtctataactactgttttaaatttatcagtgttttctgataggtaatcataagcctcgtatatgtcatcaaaactctttagactaaatacttgtatatctcctcttttaactctaagcttgtttctagctgatagagtacctttgtcctttacatcaataaagaatattggtttgggtagtgttcctgagatagtagttttacctgaaccagatcttccataaagtgttagtattgtgggctcatctatatcatatagatccactaatctgtcctcaaaactatttgattttgatttttgcttttttgccattgtcactttcctccctttgtttgtagtcagccttaataataaattctttatcaagatttaaaagttcagcttggcataaagatttatattcacagaaagagcaaccttttccaaggttcttttcctttcttttgtggccctcatctctaataagtttagctatctcaatagtatcaatcattacactgttaagtatattctttgataatattattgggtgtcttacaaagaagtcttcccatctagcagaattaatataagactcataatctttaggatctaatcctaattctcttattcctctttctaactctaggggtgtggatttaatcctcttttgagataatacccctttttgagttaattctggtctacctggttgctgagctaatattatatcccatatagtaccacttacttttgggtattcatgtagaagagcccaggtatatatagcagattgtctattgaagatcaggaaatttctatcaggcatctttttgtaggttttagtttccttagcccatatctttccatccacatctaagacactatcaatatagccttctagagttacacccttacatagttttaattcgaagtgatgttcattttccacataggttacattatcttctttttcatcataatagtggaaatagttatcacataaagaataaaccatttttggaatatctccaaattcaaggatctcttctttaaatgtatttttgtaaaactctttggaaaatttatcaacagattttttccaactcttcccattatggtagtcttctatagcctggtggatagcagagcccctttgtaaggcagctccacttcttttaggtaccagaccttcatagtatttaacataatgggcataaggacaagacaagaatttgttaattctggaattacttatttttaacatccttatacctccttttcattacaatatttatattatcagataattattcatctgtcaacacttttcttatctggcttttccaatcacctttaaaatccagttcaacacatcctccccaagaataaccaactgatatatccatgattattgggactgttggggtaaatttaaatactttctttaatactttattattttcaactattgattttactttccaagctaattcttccacatagtctttatctacttcaaataatattgagtcatgtactgagcctaatacatcaaacttagacttatctaatacatattcaggattaacatatttagcatagcctgtaatctcacataggcctaataaagtgatatctgaaccaaaaccttgaactggtgagttaatacattgtctttcggcttcagcagctttagatctatcagatgaatatatatcgggtaatcttctaattcttcctattagagatcttacttcaccattggctttaacaatttttctttgtttatcatgccatgttaatagtttagggtatttattaaagaagttccttctatatgttttggcttcctcatctgttaatttaagaccatagttgtctcttccataatccttgaattttttccattgcataccatataagaaaccaaagtttacagccttagcctttttccttttctccttcttaactgctggatctttctcatcattgatatcttccccagatataatattatatgtggagtcatgtatatctccaccagtctggtaaataaacttcatattatcctcatcggccatcatagcagctattctaagttcggcctgggatagatcggcttcaatgaatactcttccaggagatggtcctaataaactcctgattttcttatctctaggaacttgctgtagattaggattattacttgaggttcttcctgttacagttccatgaagtttaaagtttggatataatctatgattgtgcatcctatttagccaaccatctataaagtgggaaatttgtatatgaactcccctatgctgtaatagtagttctactgctggatgtttatctcttagtcttaataatacactttctccagtagctggtgctccagagtcagtaacctcaatcacaggaagaccaagtatatcatataaaaattctccaacctgtttaggtgagctccagttaatatcctggccattagtatacttcttaagtccagtctcaatcttatctagttcagatcttaagtatttttcaacctctttgaatttctcctgatttacatatatacccttgaactgaacatcctcataagctttactagctgggatgtataagtggtggaatagtttatataagctctcatcccttttaagtcttttattaaatattttatatagagcaaatgtatagtatatatcataccccagatacctaacataatcctcaaagtctgatttagtctccacatttccagtctttaatttcttatttatatcccagtctttagcattacaatgtaataaagcattctccttaagaccattaggagtattctcatctaaacaatgtgaggctagtaaagtatcaaaggttatgattggcttaataccatatttctcctttaagaaattatcatcaaacttaccattctgggctattctttccttcatctcagaattaagtcttttaatcaaggatttagctaatcttctttgtgctatgggcttaccccttaatgggctatatttgacttctaaaggcagtatatactgtacttgggtattaccaaaaccaaatagagtaatgttattattaaacctatctaagcctctagtttctatatcatatgatactctattataaccctcatcccttaaatatttgaaagcctggtttagttctttcatactagtaataagttttatgttaagatcaggtaattcatgctctttaccttttaccatggctttaaagttattaaaggcctgatctacaaattgtgctttagttgggtcatatgcaactacaccgggtgaatagctggcaataaacttaaagccatatttctcatgcttcttaggtactccacatattgaagttataccttcattacttagcatctttaatgcttgagatcctaagatcataacatattcgggtttatatttttcaatttccttaagtaaatgttcttggcatttcttaatctctgatactttgattttagtacccttaggagttctacacttaatagcattggtataataaaagtctagaccttccattttatcaagtaatgatttatcaggagtagctattctattggcctcatccctatcattagctaaactatttatgaccattattcttggcttctttttctttcctacacaagttccttctatacatgagggagctgagtgagtatataggttacagttgttacatctcatttaaaatattacctcctaaatagaaaggacccctaaaggcccttatctttattttatgattgagttacatactggacagaccttatgttttttgaagggtatggttactacccataggcctccagttaagaaaatcatgatccaaaacatagctccatattttctttttaatgttactgagtttttacacataggacaaattatatttttcattaggatagccccctttaaatttagaatatcatatgatatattatattggcaatatcaaaaattattacccataatcctatagctgctaagattataattaaacaaccaagacagccattgttattgttcttaggtctgttatcatcactataattatacatattacttactccacagttcatccatataatttatatagttattaagttcattcctagtcatgtccccaaggttagctggttctaaatcaaattccttttcagtattcctaataaattgctttagggtttccttcttgttaaccttattattaagatcagaatgtttatatctttcttttctcatgtaactcatttattagaatacccccttaatatctttgttgtaaacatgaagagagaaaattgtatgagagaaacttcctggttcatagccagtttgttcagctacccaatgtaatagtttcatagcaagataaacatcattagcaaagtgagtagcaaaatcagaacttctcataacataatggatatttagcttaccttctcttacttggaagttatatcctaatgaacatggtactctagttactcctcctatattgaatggatcaatagctggattccacagagataaccataattgtcttgagcctggatcttctttaattctattgatgatatcctcaatttgtctgtattgccaaattctttcattgtaagaatacccaaattttccatctcttagatattcattccatacctcaggtcttaattgataagctttaccaggatttatgaaagcctccctagtatgatgtggatgtataccaaataattcttctctttcttcaagagagtattgattgatgacaccttgtggatcgtagatcctttctctaaattcagcatctgcccaaggttgagatacacctggaacttcttcaggtttactttctagaattgtgtaactatagttttgtaactcctttgtgaaataatctggattaccttctataactttatcttgcatagttttgggtcttaccccaatccccatttcacataaatctctttttacttcttcaaatgcttcttgagcattaatataaattctcatagtttaattcctccatttatttaattttgttaagttaattatactacttattaaagtacttgtcaatagataatttattgatatctatctttggaaatttctccagaccaaaatgtaataactgcatcttctggagagctttataagagtgtatctggtcctctgatttaaagaacctgttatagttactattcaaggatttatgccaaggatgtttgctattagcaatactctttcttggtaccttaaaataattgaaatatccatttataaacattcctgacaaataagcttgagacatatgaaaagtaatattatctatctcacatacttcttgaggtagttcttcaatgaacctgtttattaatactagatcagctgcgaatttcttttgtaattcacatactctatacataatttttaagtgtttccaaggtccttttctttttggtctagttactactgcagctatcaagcaagaaccattagtagcttttttcctgttgaaataataagtatagctcataccacttatcttggtaagcttttctctaaattcaattaattgtggataatcaatgtatgatcttaataggtgtccccacttaccttctttatatccaaagtcccctagatttaaagtacatttatgggacttacaggagagaactaagtcctcctgaaagccctgtatgttctgagtatacatcatagtttcttctggattggtaatcatttccctattaaggtttaagaataagtcatcaaaatcattatagtctcttattagcatattaccttctcctaagtatttattttagtaattagatctttggcggaatttatttacctgtgatttcttaaggtatatatttactatgtcatctacctctaagccagatacagctaataatttaatgtaacatacccatacattgaataatctttgattaaaagcatttacatctgttagcattgaagtttgtttccaaggtttattcttaaggcagttacagcacatacccatttctcttaccaggtcagttacagcttcttctactaacatttcaggaaattctggtgatgtagtagccttatgatataagttctctaggctatcaactaatatagcattattatctatagtattataatccttaccagctagaattgtaaattcagttaagaagtgtaatccatcaattaattcttcttggtaatggtcttcatgattataagcatccaatgcttctcctacttcttcagtcattctccaagcaaaatctttaagtctagcttgacctcttttatcatttaagttaactggacagtcttcagtttggcataatcctgatctagcttctatatgatgatatttctccattaactccttttgtctattaaagatagcttgtaatctatctccttctattttttcttctactgcatggtttatattcataacaatctctcctcttatcttgatatatttataaattggtttatagcttctttagcacttgagtcatctattaactgggatagcttctccacattggaagtagtataatcatataccagtacattccatccatcacagaataacttccatatcagttcatcatatctagccagtagatgttcagctctttcaattactcctggcatctgttctctatcaccaaaattgaagatcacttccctaggtggtctagcatatacaatagttggcttacatagatgttttaagatctttagctccttactgtcaaggttgaaattactactatctctgatgataggtccatacaccatttcttcaaagcaagtaaatctatcatgtatagcttccctttcaccttttctcacaatttgagttaatacccattctctttgttcttcataagaaccaggtcccattgattggatatattctcctcctctgtgtttagttaggttcttagctgttgtggtcttacctgagttatccattcctaaaatgataatcattaaagctctcctccattctttagatcttctactattaagtttagtatatattgtactcctttatcattatattcaaataaaggatttataagggacttacttggagttacataataaccaagttctttagcaaggattgggtctattatctcaagtgtatgctcattgtaccttctggcaaatccctttcttactaaatacctatttagttttatcacactaactcctaatgctcctgctatcttagtagcagtggttaaacttcccttccatagttggggtttgtcatcattaaggtctttcaagatgtaatactttttattgaccattaaattctcctccttctacatttttatattaccataattaatttattatgtcaaaggttattttagaatttttaggtatatctataacagccagaagattttctggtctattactatcataaacaagtatagtataattctgagctcctaagttattgaccataacctcattagctaacttagataagttgttaggggtaaggtctttaggactattaaggtttagtttgataataagatcctccccatctagtccagatggagaagtctcaataacattatagtctaaagcattatgaagcttttctactaacttttcttgactttttctttggtgatgactttctattagttttgccccctgagttagcattatccccattgacaatgatatccctaggattagtattacttccttcaagtttcttcttcgcattagccttagcctccctatatcttatattcatacattttacataaaagtcttggtcacttataccacagatagggcaattcttgtaacctccttggcttctcttaaattcttgaatagtttgacaatatggacaccacattttcttcttaggtatctcttcgccttcagggatcttatgggcttcatggacatccacccaataaaattcagcccagggacattcttccataactttgtctataaataatttagctgatttataggtatagaaatatttcaatcctgaatgataagtgattttattcttcttacctctagcaataattactactacaaaggcctttatatgattatgacctgctggcctcttacactttattatcatgcctttttcctcccaatatttagtttcttacttatattataacctttatccggagaatatacaatagtatcttttaaagtatctagaactggattaaccttctgtgaatttaatcctgatattgacactatctcctccttggtatgagctcctgattttacagcctctataactttggctttgtcctcaggtttcacaattacttcttttctgggtattgctacttctacatgataatatggatctccaaattctcccattgataaattcaattcaatttgagggaattgtcctgcaagacggaactctctatccataatgattttacttggtaaatggctttgtttatcaaggttatctatatctacttcaatctcctcatcgtcaccttctaagtcatcaggtctttttaaatataatgctgattctacccaaccatgtaatatgaatgaaccagccatcttttgaccacctctggtttgagtggcatttccacctttattatagtggtgtattaacataactcctgtatgcttctcattcttaagtttaagacaccattgtagtacaggattaagatcagctgcattattaagatctcccctaaacataagatataatgggtcgaatattactagtacaggttttatctcatcaattaattcttctatctgttttctatgggattcttcatctaacataaatccctgttgattaataaaagtgataggaagatctggagcaaacctaactttaagtcttctcttaccctttatatccacattaccaactactcctctgtggctaattatcttttcagttctatccctcataatccagtcagcattctcattttgaactacaattactgggcctggttctagaacaggatattgacctaggaagggtcttccactagcaactgatatagctaagtcctgtgtaaatgtggatttaaatacctttggttgtccagccacaattccatgagatcttctaccccagaaaccttgtactaaccaacctgggaaggcaccattattacccataacatcctgataactatctattctcagtttagtactttcagccttttcaatatcagcctctatttctcctcctatgattttatccaattcttttcttaaccttgtttcttcatcttttcttcccttatatttattaaaagctgagcccttaactaataatataatctcattaggctctagtcctatttcatgtaatttattctcaatataccatatagtagaacttctatctaaagaagtaatgtcatctaaagccagtaagtctctaaccttctttggtatattatatttagcatatatctttctttcagattgtgaggcctcagatcctcctatattgaccttaacactatcattagatttacttacagccttaacagccttagcgatcaccttaggcttatatatctccttagtgtgtataggtctttttacttttggtttattcttgtatttatagttaatagttcctggtattctatatacatgagtaacatcaaagcaggagtcacagcctatatgtttagctaatgctggatttatttcgtcatattgattagcctctatatacctatccatttcccatagcccctgatattttccaggagaactttcccacagataacttggtttaggtttaatccccaatgggtcagtatgctcatctatatcttgtattaagtatttagtctctatgaagttaactatccttctttgaggattactatagggcattgggctccaatataaatcataacccttatactgttgttcaaagtcctttagttttttgtcaatgttattcttattatatttgattggtacatctttccattctttaccttttctagctgctaggataatgtaatctctattttcacattgtttagagaatatatccttcaagaactttatgtccatatattataccccctattataagtctatattatcccaacctaattctttcaagtatggaactacttctcctcttggctttaattttctagtgccttcctctatctcagcgaatactaatccccctatatgtggtttagtcccgttaactactctcattatactaacagccgatactcctaactgtttagctgcatatctgaaggatctatactccctattattgttgtaacaatatactgctttagtataagttgaatttccacctcttgccatttatacatccccctctaacatctgtttctaaaataagtaaaaaatttgaggagcaagtttgctccccttattatttgatgagaattattcttcatcatcagcttctaataattcaattatctcagctggtttcattttcttattaacttttattcctctttctttagcaagagcaattaagtctttcttagtcatttcagagtagtcaggagtttcatcctcttcttcttcctcttcgtcttcttcttcaccttgagcttctttgattaaagcgattaactcatctttatcttttttcttagctcctttgatacctaagtctttagccatagcagctaattcctttttagataatgattctaaatcattttcatcttcttcttctgcttcgtcttcatcaacttcttcgaagtcagcatctactacaccttcatcttccacagcatctatttctgcttggtatgcagcctttacagttcctacagccatttctaatgattctaatgcttcctctacagttatttgtccatctgtgtcaggagttctttcatctaattccacaatagcttttaaagcctttttaacttctttctcatctccagaatttaaagcagattgtacgattacaattagctccttattgtttgcttcctctaaccattttgcttttccttttgccataataatcattcctccatatttttaatttttaaataacaaatttagtatagtttgaaattaactaattataaagttttggttggtgtttgtaatttgattacaatactataatatcatatcctatatagcctgtcaacgagttatttagaaaaaattaatttattataacattcattacaaacggcttcatattcaacactttcgggctggttatcaatttgtatctggttaccctggtcagtatatttaccctggtattttaatattgagaatgtggcttttttaccacattgacaaatgttctttaattcttcaatattatgggccacttgtaataatctggtacttccttcaaatccttcccttttaaagtcagttctcaatccataacatataataggataatgtaatgataaatttaacagatcatcaacctgttctctggataagaattgtacctcatcaattaatataacatctactgcccaataattagactcaaagtcagaaagtatttttgataatttaactctaggaggtagaagaacatccacctttcttgctacccctattctactgattatacatggtccacctttagtatcaattccgggcttaactactaatggcttcattcccctttcttcatagttatgtgctacctggattaactgagtagtctttccagagttcatagcactatacctaaaatataacttattgctcacaactgatcgcctccattatacaccatactattacaagtatgcctaatattctaaatgcccataataaatatcccaatactatcactcctttgactcctcccctaaatcaaatatacctggtggtactaaatccttaatctctcccattatggtttcatagttaagtgttcccttttcaatctcctctgtgtgtttactcatcccttccacaaacctagtcattctagtcttaccataaccttccttctttaatgtatagcatgataaggctaacatgatgtccacagctttaagaacattaagatttttgttctctctttcggctcttctccttgcagctcttgctcttgacataataatctactcctttatatatttagtttctaaaaatattgatactattatagctagtatcgcaaaacctagttccatttcttcacctcaaaacctataaacactcctagtaaaaatattgatactagggttattacccctagcaccatttacttctcctcccataacaggtcagaataatcagttccttggtcatatgagaatattaaacctttctgtgaactgatataatcagccaagtgtactattctctgggaataactattaataggaacactaccccattgaccatgatgagactcaattagttcaactaccactttgtatattattggaaactcttcctctaggggtgatagtgtctctctaaccatatatggatgttctttatctggcttattaatgtcatgtaatattaaagcagctattatcatatctctgtcccttgaacatatcatctcagcttcgcataatgctttacctatataacaagcagctttagtatgtcttaacaaacctcctacccctgcactataagttggatgatatttcccagtactacttgcaggtattataaagaacttttcatcaactatctcatttagggcctttcttacaaaattttgtatatccctatcttttatatcatgtatttctggtattagcattctcatgcccatttctcttatcataactattcctcctatcccatgtagtagcctctatattttatcttctcccactcatcaacagtaaataccatcttcactctttgtggtgtattagaataacaaatatagtccatgtctacttctacatattgtttacctttagcccaaggttcattatcaaattcatggtactctcttacactgtgtaccttttttatatagtgctcaagtaggttcatttctttttcctcctcttcttcttctttttcttactctttccatcaagtcctcgtttaacatgaaagtcaagtaagttttgagcccaccttaacatcttaatatcttgcatacatgaaaggttaaagccagtggatccatcaaagactttaaggtcattcctaaatggcatactgtttactaaacctggattctcattcttaagtttaactacctctctggcagtctcatcccattgttggtctgtccagatattgttgtcatatctataatatattattgaatgaagacaaatctgtaaccacttctttcgtaattcaatcctttctggagtttcttcgcagtcatacttgagaattaacatagcacttcttctccccaatattatcacctccttttctattataccatattcttttaccttctacaatagaaaaagtttgaccaatatgttctggttcaatttcctcaatggtaagtgttcccccatgcttacatagtatcttagctaatacttgtcccatgtctgtatctgctaaagataccccactattttttctggttattacatacgacttcataacttagccccactctcaaatttattaactgattatttatctcttgtatttcttttaacttcttctcagtcaatcctaagaactgtcccaattttatcttctgttcttttgttaaatgacaatactgtttctcaatcaaatatctggcatagtttaggttctttcttatctcatcagtattttgattatgcttttctctatcccttccagtctcttcaataatgatgtgtttatcatgtgatacctccctaataagatattttgttatctttggctttctgtcactaaagtccattactgtagctacatccccatcga